European Patent Application EP 4 733 395 A1, published April 29, 2026. Title: Cas12j PROTEIN WITH ENHANCED EDITING ACTIVITY AND USE THEREOF. Applicant: SHANDONG SHUNFENG BIOTECHNOLOGY CO., LTD. Application CN. The sequence listing filed with the application follows.

SEQUENCE LISTING (2 sequences)

SEQ ID NO: 1 - protein, 908 aa, synthetic construct
  REGION 1..908: note = Cas12j19
MPSYKSSRVLVRDVPEELVDHYERSHRVAAFFMRLLLAMRREPYSLRMRDGTEREVDLDETDDFLRSAGCEEPDAVSDDLRSFALAVLHQDNPKKRAFLESENCVSILCLEKSASGTRYYKRPGYQLLKKAIEEEWGWDKFEASLLDERTGEVAEKFAALSMEDWRRFFAARDPDDLGRELLKTDTREGMAAALRLRERGVFPVSVPEHLDLDSLKAAMASAAERLKSWLACNQRAVDEKSELRKRFEEALDGVDPEKYALFEKFAAELQQADYNVTKKLVLAVSAKFPATEPSEFKRGVEILKEDGYKPLWEDFRELGFVYLAERKWERRRGGAAVTLCDADDSPIKVRFGLTGRGRKFVLSAAGSRFLITVKLPCGDVGLTAVPSRYFWNPSVGRTTSNSFRIEFTKRTTENRRYVGEVKEIGLVRQRGRYYFFIDYNFDPEEVSDETKVGRAFFRAPLNESRPKPKDKLTVMGIDLGINPAFAFAVCTLGECQDGIRSPVAKMEDVSFDSTGLRGGIGSQKLHREMHNLSDRCFYGARYIRLSKKLRDRGALNDIEARLLEEKYIPGFRIVHIEDADERRRTVGRTVKEIKQEYKRIRHQFYLRYHTSKRDRTELISAEYFRMLFLVKNLRNLLKSWNRYHWTTGDRERRGGNPDELKSYVRYYNNLRMDTLKKLTCAIVRTAKEHGATLVAMENIQRVDRDDEVKRRKENSLLSLWAPGMVLERVEQELKNEGILAWEVDPRHTSQTSCITDEFGYRSLVAKDTFYFEQDRKIHRIDADVNAAINIARRFLTRYRSLTQLWASLLDDGRYLVNVTRQHERAYLELQTGAPAATLNPTAEASYELVGLSPEEEELAQTRIKRKKREPFYRHEGVWLTREKHREQVHELRNQVLALGNAKIPEIRT

SEQ ID NO: 2 - RNA, 2724 nt, synthetic construct
  source 1..2724: mol_type = other RNA
  misc_feature 1..2724: note = Cas12j19
atgcccagctacaagagcagcagagtgctggtgagggacgtgccagaggagctggtggaccactacgaaagaagccacagggtggccgccttcttcatgagactgctgctggccatgagaagagagccctacagcctgagaatgagggacggaaccgagagagaggtggacctggacgaaaccgacgacttcctgagaagcgccggatgcgaggagccagacgccgtgtctgacgacctgagaagcttcgccctggccgtgctgcaccaggacaacccaaagaagagagcctttctggagagcgagaactgcgtgtcaatcctgtgtctggagaaaagcgcctccggcaccagatactacaaaagacccggctaccagctgctgaagaaggccatcgaggaggagtggggatgggacaagttcgaggcctctctgctggacgagagaacaggagaagtggccgagaagttcgccgccctgagcatggaagactggagaagattcttcgccgccagagaccccgacgatctgggaagagagctgctgaagaccgacaccagagaaggcatggccgccgccctgagactgagagaaagaggagtgttccccgtgagcgtgcccgagcacctggacctggacagcctgaaggccgccatggccagcgccgctgaaagactgaagtcatggctggcctgtaaccagcgcgccgtggacgagaagagcgaactgagaaagagattcgaggaggccctggacggagtggaccctgaaaagtatgccctgtttgagaagttcgctgccgagctgcagcaggccgactacaacgtgaccaagaaactggtgctggccgtgagcgccaagttccccgctaccgagcctagcgagtttaagagaggagtggagatcctgaaggaagatggctacaagcccctgtgggaggactttagagagctgggctttgtgtatctggccgagagaaagtgggaaagaagaagaggcggagccgccgtgaccctgtgtgacgctgacgacagccctatcaaggtgagatttggactgactggcagaggcagaaagtttgtgctgtccgccgccgggagcagattcctgatcacagtgaagctgccctgcggcgatgtgggactgaccgccgtgcccagcaggtacttttggaacccctcagtgggcagaaccacctccaactcttttagaattgagttcaccaagcggaccaccgagaatcgcaggtacgtgggcgaggtgaaagagattggcctggtgaggcagagaggcagatactattttttcatcgactacaacttcgacccagaggaggtgagcgacgagaccaaggtgggcagagccttcttcagagcccccctgaacgagtcaagacctaagccaaaggacaagctgaccgtgatggggattgacctgggcattaacccagcctttgcctttgccgtgtgcaccctgggcgaatgccaggacggaatccggagccccgtggccaaaatggaggacgtgagcttcgactctaccggactgagaggcggaatcggcagccagaagctgcacagagagatgcacaacctgagcgacagatgcttttacggcgccagatacattagactgagcaagaagctgagggacagaggagctctgaacgatatcgaggctagactgctggaagagaagtacatccccggctttagaattgtgcacattgaggacgccgacgagagaagaagaaccgtgggaagaacagtgaaagaaatcaaacaggagtacaaaagaatcagacaccagttctacctgaggtaccacaccagcaagagggacagaacagagctgattagcgccgagtacttcagaatgctgttcctggtgaagaacctgagaaacctgctgaagagctggaacagataccactggacaaccggcgacagagaaagaagaggagggaacccagacgagctgaagagctatgtgagatactataacaatctgagaatggacaccctgaagaaactgacctgcgccatcgtgaggaccgccaaggaacacggagccaccctggtggccatggagaacatccagagagtggacagggacgacgaggtgaaaagaagaaaggaaaatagcctgctgagcctgtgggcccccggaatggtgctggagagagtggagcaggagctgaagaacgagggaatcctggcctgggaggtggacccaagacatacaagtcagacaagctgcatcaccgacgaatttggctacagaagcctggtggccaaggacaccttctactttgaacaggacagaaaaatccacagaatcgacgccgacgtgaacgccgccatcaacatcgcccgccgcttcctgacccggtacaggagcctgacccagctgtgggccagcctgctggacgacggcagatacctggtgaacgtgaccagacagcacgagagagcctacctggaactgcagaccggcgcccccgccgctacactgaaccctaccgccgaagccagctacgaactggtgggactgagccccgaagaagaagagctggcccagaccagaatcaaacgcaaaaagagagaaccattctacagacacgaaggcgtgtggctgacaagagagaagcacagagagcaggtgcacgaactgagaaaccaggtgctggccctgggcaacgccaagatccccgaaatcagaacc